European Patent Specification EP 3 972 593 B1, published July 2, 2025. Title: INHIBITOR OF MNK FOR THE TREATMENT OF NEUROPATHIC PAIN. Applicant: BOARD OF REGENTS, THE UNIVERSITY OF TEXAS SYSTEM. The sequence listing filed with the application follows.

SEQUENCE LISTING (12 sequences)

SEQ ID NO: 1 - DNA, 21 bp, Artificial sequence
  Synthetic primer
cccggaagacagatagcctga

SEQ ID NO: 2 - DNA, 23 bp, Artificial sequence
  Synthetic primer
ttcaatggcaatgtgtaatgctg

SEQ ID NO: 3 - DNA, 20 bp, Artificial sequence
  Synthetic primer
ggctgtattcccctccatcg

SEQ ID NO: 4 - DNA, 22 bp, Artificial sequence
  Synthetic primer
ccagttggtaacaatgccatgt

SEQ ID NO: 5 - DNA, 22 bp, Artificial sequence
  Synthetic primer
tcatacttcggttgcatgaagg

SEQ ID NO: 6 - DNA, 19 bp, Artificial sequence
  Synthetic primer
agacctctcgaacctgccc

SEQ ID NO: 7 - DNA, 19 bp, Artificial sequence
  Synthetic primer
gcgtggatgccatgacaac

SEQ ID NO: 8 - DNA, 21 bp, Artificial sequence
  Synthetic primer
aatgatgagcacttcgtccct

SEQ ID NO: 9 - DNA, 20 bp, Artificial sequence
  Synthetic primer
gacaactttggcattgtgga

SEQ ID NO: 10 - DNA, 22 bp, Artificial sequence
  Synthetic primer
catcatacttggcaggtttctc

SEQ ID NO: 11 - DNA, 20 bp, Artificial sequence
  Synthetic primer
acgtccgattcttggggaac

SEQ ID NO: 12 - DNA, 20 bp, Artificial sequence
  Synthetic primer
tacggaagatgttgtcccgc